European Patent Specification EP 4 023 751 B1, published March 11, 2026. Title: Novel acetohydroxy acid synthase variant and microorganism comprising thereof. Applicant: CJ CheilJedang Corporation. The sequence listing filed with the application follows.

SEQUENCE LISTING (78 sequences)

SEQ ID NO: 1 - protein, 626 aa, Artificial Sequence
  acetohydroxy acid synthase, AHAS
MNVAASQQPTPATVASRGRSAAPERMTGAKAIVRSLEELNADIVFGIPGGAVLPVYDPLYSSTKVRHVLVRHEQGAGHAATGYAQVTGRVGVCIATSGPGATNLVTPIADANLDSVPMVAITGQVGSGLLGTDAFQEADIRGITMPVTKHNFMVTNPNDIPQALAEAFHLAITGRPGPVLVDIPKDVQNAELDFVWPPKIDLPGYRPVSTPHARQIEQAVKLIGEAKKPVLYVGGGVIKADAHEELRAFAEYTGIPVVTTLMALGTFPESHELHMGMPGMHGTVSAVGALQRSDLLIAIGSRFDDRVTGDVDTFAPDAKIIHADIDPAEIGKIKQVEVPIVGDAREVLARLLETTKASKAETEDISEWVDYLKGLKARFPRGYDEQPGDLLAPQFVIETLSKEVGPDAIYCAGVGQHQMWAAQFVDFEKPRTWLNSGGLGTMGYAVPAALGAKAGAPDKEVWAIDGDGCFQMTNQELTTAAVEGFPIKIALINNGNLGMVRQWQTLFYEGRYSNTKLRNQGEYMPDFVTLSEGLGCVAIRVTKAEEVLPAIQKAREINDRPVVIDFIVGEDAQVWPMVSAGSSNSDIQYALGLRPFFDGDESAAEDPADIHEAVSDIDAAVESTEA

SEQ ID NO: 2 - DNA, 1881 bp, Artificial Sequence
  ilvB variant n.t
gtgaatgtggcagcttctcaacagcccactcccgccacggttgcaagccgtggtcgatccgccgcccctgagcggatgacaggtgcaaaggcaattgttcgatcgctcgaggagcttaacgccgacatcgtgttcggtattcctggtggtgcggtgctaccggtgtatgacccgctctattcctccacaaaggtgcgccacgtcttggtgcgccacgagcagggcgcaggccacgcagcaaccggctacgcgcaggttactggacgcgttggcgtctgcattgcaacctctggcccaggagcaaccaacttggttaccccaatcgctgatgcaaacttggactccgttcccatggttgccatcaccggccaggtcggaagtggcctgctgggtaccgacgctttcaacgaagccgatatccgcggcatcaccatgccagtgaccaagcacaacttcatggtcaccaaccctaacgacattccacaggcattggctgaggcattccacctcgcgattactggtcgccctggccctgttctggtggatattcctaaggatgtccagaacgctgaattggatttcgtctggccaccaaagatcgacctgccaggctaccgcccagtttcaacaccacatgctcgccagatcgagcaggcagtcaagctgatcggtgaggccaagaagcccgtcctttacgttggtggtggcgtaatcaaggctgacgcacacgaagagcttcgtgcgttcgctgagtacaccggcatcccagttgtcaccaccttgatggctttgggtactttcccagagtctcacgagctgcacatgggtatgccaggcatgcatggcactgtgtccgctgttggtgcactgcagcgcagcgacctgctgattgctatcggctcccgctttgatgaccgcgtcaccggtgacgttgacaccttcgcgcctgacgccaagatcattcacgccgacattgatcctgccgaaatcggcaagatcaagcaggttgaggttccaatcgtgggcgatgcccgcgaagttcttgctcgtctgctggaaaccaccaaggcaagcaaggcagagaccgaggacatctccgagtgggttgactacctcaagggcctcaaggcacgtttcccgcgtggctacgacgagcagccaggcgatctgctggcaccacagtttgtcattgaaaccctgtccaaggaagttggccccgacgcaatttactgcgccggcgttggccagcaccaaatgtgggcagctcagttcgttgactttgaaaagccacgcacctggctcaactccggtggactgggcaccatgggctacgcagttcctgcggcccttggagcaaaggctggcgcacctgacaaggaagtctgggctatcgacggcgacggctgtttccagatgaccaaccaggaactcaccaccgccgcagttgaaggtttccccattaagatcgcactaatcaacaacggaaacctgggcatggttcgccaatggcagaccctattctatgaaggacggtactcaaatactaaacttcgtaaccagggcgagtacatgcccgactttgttaccctttctgagggacttggctgtgttgccatccgcgtcaccaaagcggaggaagtactgccagccatccaaaaggctcgagagatcaacgaccgcccagtagtcatcgacttcatcgtcggtgaagacgcacaggtatggccaatggtgtctgctggatcatccaactccgatatccagtacgcactcggattgcgcccattctttgatggtgatgaatctgcagcagaagatcctgccgacattcacgaagccgtcagcgacattgatgccgccgttgaatcgaccgaggcataa

SEQ ID NO: 3 - DNA, 23 bp, Artificial Sequence
  primer
attctagaggccaagaagtccgc

SEQ ID NO: 4 - DNA, 29 bp, Artificial Sequence
  primer
cttgttgctgctacacacatcgagtttcc

SEQ ID NO: 5 - DNA, 29 bp, Artificial Sequence
  primer
tgtagcagcaacaagattttggcaaaatg

SEQ ID NO: 6 - DNA, 23 bp, Artificial Sequence
  primer
attctagagccgaacggcgcccc

SEQ ID NO: 7 - DNA, 1881 bp, Artificial Sequence
  Corynebacterium glutamicum ATCC 13032 hom/ilvA variant
gtgaatgtggcagcttctcaacagcccactcccgccacggttgcaagccgtggtcgatccgccgcccctgagcggatgacaggtgcaaaggcaattgttcgatcgctcgaggagcttaacgccgacatcgtgttcggtattcctggtggtgcggtgctaccggtgtatgacccgctctattcctccacaaaggtgcgccacgtcttggtgcgccacgagcagggcgcaggccacgcagcaaccggctacgcgcaggttactggacgcgttggcgtctgcattgcaacctctggcccaggagcaaccaacttggttaccccaatcgctgatgcaaacttggactccgttcccatggttgccatcaccggccaggtcggaagtggcctgctgggtaccgacgctttccaggaagccgatatccgcggcatcaccatgccagtgaccaagcacaacttcatggtcaccaaccctaacgacattccacaggcattggctgaggcattccacctcgcgattactggtcgccctggccctgttctggtggatattcctaaggatgtccagaacgctgaattggatttcgtctggccaccaaagatcgacctgccaggctaccgcccagtttcaacaccacatgctcgccagatcgagcaggcagtcaagctgatcggtgaggccaagaagcccgtcctttacgttggtggtggcgtaatcaaggctgacgcacacgaagagcttcgtgcgttcgctgagtacaccggcatcccagttgtcaccaccttgatggctttgggtactttcccagagtctcacgagctgcacatgggtatgccaggcatgcatggcactgtgtccgctgttggtgcactgcagcgcagcgacctgctgattgctatcggctcccgctttgatgaccgcgtcaccggtgacgttgacaccttcgcgcctgacgccaagatcattcacgccgacattgatcctgccgaaatcggcaagatcaagcaggttgaggttccaatcgtgggcgatgcccgcgaagttcttgctcgtctgctggaaaccaccaaggcaagcaaggcagagaccgaggacatctccgagtgggttgactacctcaagggcctcaaggcacgtttcccgcgtggctacgacgagcagccaggcgatctgctggcaccacagtttgtcattgaaaccctgtccaaggaagttggccccgacgcaatttactgcgccggcgttggccagcaccaaatgtgggcagctcagttcgttgactttgaaaagccacgcacctggctcaactccggtggactgggcaccatgggctacgcagttcctgcggcccttggagcaaaggctggcgcacctgacaaggaagtctgggctatcgacggcgacggctgtttccagatgaccaaccaggaactcaccaccgccgcagttgaaggtttccccattaagatcgcactaatcaacaacggaaacctgggcatggttcgccaatggcagaccctattctatgaaggacggtactcaaatactaaacttcgtaaccagggcgagtacatgcccgactttgttaccctttctgagggacttggctgtgttgccatccgcgtcaccaaagcggaggaagtactgccagccatccaaaaggctcgagagatcaacgaccgcccagtagtcatcgacttcatcgtcggtgaagacgcacaggtatggccaatggtgtctgctggatcatccaactccgatatccagtacgcactcggattgcgcccattctttgatggtgatgaatctgcagcagaagatcctgccgacattcacgaagccgtcagcgacattgatgccgccgttgaatcgaccgaggcataa

SEQ ID NO: 8 - DNA, 31 bp, Artificial Sequence
  primer
tccggatcctgacacaccatgaccattattc

SEQ ID NO: 9 - DNA, 30 bp, Artificial Sequence
  primer
tccggatcccttatgtacaaagtgcacagc

SEQ ID NO: 10 - DNA, 25 bp, Artificial Sequence
  primer
cttcgttgaaagcgtcggtacccag

SEQ ID NO: 11 - DNA, 25 bp, Artificial Sequence
  primer
ctttcaacgaagccgatatccgcgg

SEQ ID NO: 12 - protein, 626 aa, Artificial Sequence
  acetohydroxy acid synthase variant
MNVAASQQPTPATVASRGRSAAPERMTGAKAIVRSLEELNADIVFGIPGGAVLPVYDPLYSSTKVRHVLVRHEQGAGHAATGYAQVTGRVGVCIATSGPGATNLVTPIADANLDSVPMVAITGQVGSGLLGTDAFNEADIRGITMPVTKHNFMVTNPNDIPQALAEAFHLAITGRPGPVLVDIPKDVQNAELDFVWPPKIDLPGYRPVSTPHARQIEQAVKLIGEAKKPVLYVGGGVIKADAHEELRAFAEYTGIPVVTTLMALGTFPESHELHMGMPGMHGTVSAVGALQRSDLLIAIGSRFDDRVTGDVDTFAPDAKIIHADIDPAEIGKIKQVEVPIVGDAREVLARLLETTKASKAETEDISEWVDYLKGLKARFPRGYDEQPGDLLAPQFVIETLSKEVGPDAIYCAGVGQHQMWAAQFVDFEKPRTWLNSGGLGTMGYAVPAALGAKAGAPDKEVWAIDGDGCFQMTNQELTTAAVEGFPIKIALINNGNLGMVRQWQTLFYEGRYSNTKLRNQGEYMPDFVTLSEGLGCVAIRVTKAEEVLPAIQKAREINDRPVVIDFIVGEDAQVWPMVSAGSSNSDIQYALGLRPFFDGDESAAEDPADIHEAVSDIDAAVESTEA

SEQ ID NO: 13 - DNA, 25 bp, Artificial Sequence
  primer
tcggcttcgcggaaagcgtcggtac

SEQ ID NO: 14 - DNA, 25 bp, Artificial Sequence
  primer
cgctttccgcgaagccgatatccgc

SEQ ID NO: 15 - DNA, 24 bp, Artificial Sequence
  primer
cggcttcgaagaaagcgtcggtac

SEQ ID NO: 16 - DNA, 25 bp, Artificial Sequence
  primer
cgctttcttcgaagccgatatccgc

SEQ ID NO: 17 - DNA, 24 bp, Artificial Sequence
  primer
cggcttcggagaaagcgtcggtac

SEQ ID NO: 18 - DNA, 25 bp, Artificial Sequence
  primer
cgctttctccgaagccgatatccgc

SEQ ID NO: 19 - DNA, 24 bp, Artificial Sequence
  primer
cggcttcgtagaaagcgtcggtac

SEQ ID NO: 20 - DNA, 25 bp, Artificial Sequence
  primer
cgctttctacgaagccgatatccgc

SEQ ID NO: 21 - DNA, 24 bp, Artificial Sequence
  primer
cggcttcgcagaaagcgtcggtac

SEQ ID NO: 22 - DNA, 25 bp, Artificial Sequence
  primer
cgctttctgcgaagccgatatccgc

SEQ ID NO: 23 - DNA, 24 bp, Artificial Sequence
  primer
cggcttctgggaaagcgtcggtac

SEQ ID NO: 24 - DNA, 25 bp, Artificial Sequence
  primer
cgctttcccagaagccgatatccgc

SEQ ID NO: 25 - DNA, 24 bp, Artificial Sequence
  primer
cggcttcgtggaaagcgtcggtac

SEQ ID NO: 26 - DNA, 25 bp, Artificial Sequence
  primer
cgctttccacgaagccgatatccgc

SEQ ID NO: 27 - DNA, 24 bp, Artificial Sequence
  primer
cggcttccaggaaagcgtcggtac

SEQ ID NO: 28 - DNA, 25 bp, Artificial Sequence
  primer
cgctttcctggaagccgatatccgc

SEQ ID NO: 29 - DNA, 24 bp, Artificial Sequence
  primer
cggcttcgatgaaagcgtcggtac

SEQ ID NO: 30 - DNA, 25 bp, Artificial Sequence
  primer
cgctttcatcgaagccgatatccgc

SEQ ID NO: 31 - DNA, 24 bp, Artificial Sequence
  primer
cggcttcggtgaaagcgtcggtac

SEQ ID NO: 32 - DNA, 25 bp, Artificial Sequence
  primer
cgctttcaccgaagccgatatccgc

SEQ ID NO: 33 - DNA, 24 bp, Artificial Sequence
  primer
cggcttccttgaaagcgtcggtac

SEQ ID NO: 34 - DNA, 25 bp, Artificial Sequence
  primer
cgctttcaaggaagccgatatccgc

SEQ ID NO: 35 - DNA, 24 bp, Artificial Sequence
  primer
cggcttcaacgaaagcgtcggtac

SEQ ID NO: 36 - DNA, 25 bp, Artificial Sequence
  primer
cgctttcgttgaagccgatatccgc

SEQ ID NO: 37 - DNA, 24 bp, Artificial Sequence
  primer
cggcttcagcgaaagcgtcggtac

SEQ ID NO: 38 - DNA, 25 bp, Artificial Sequence
  primer
cgctttcgctgaagccgatatccgc

SEQ ID NO: 39 - DNA, 24 bp, Artificial Sequence
  primer
cggcttcgtcgaaagcgtcggtac

SEQ ID NO: 40 - DNA, 25 bp, Artificial Sequence
  primer
cgctttcgacgaagccgatatccgc

SEQ ID NO: 41 - DNA, 24 bp, Artificial Sequence
  primer
cggcttcctcgaaagcgtcggtac

SEQ ID NO: 42 - DNA, 25 bp, Artificial Sequence
  primer
cgctttcgaggaagccgatatccgc

SEQ ID NO: 43 - DNA, 24 bp, Artificial Sequence
  primer
cggcttcgccgaaagcgtcggtac

SEQ ID NO: 44 - DNA, 25 bp, Artificial Sequence
  primer
cgctttcggcgaagccgatatccgc

SEQ ID NO: 45 - DNA, 24 bp, Artificial Sequence
  primer
cggcttcccagaaagcgtcggtac

SEQ ID NO: 46 - DNA, 25 bp, Artificial Sequence
  primer
cgctttctgggaagccgatatccgc

SEQ ID NO: 47 - protein, 626 aa, Artificial Sequence
  acetohydroxy acid synthase variant
MNVAASQQPTPATVASRGRSAAPERMTGAKAIVRSLEELNADIVFGIPGGAVLPVYDPLYSSTKVRHVLVRHEQGAGHAATGYAQVTGRVGVCIATSGPGATNLVTPIADANLDSVPMVAITGQVGSGLLGTDAFREADIRGITMPVTKHNFMVTNPNDIPQALAEAFHLAITGRPGPVLVDIPKDVQNAELDFVWPPKIDLPGYRPVSTPHARQIEQAVKLIGEAKKPVLYVGGGVIKADAHEELRAFAEYTGIPVVTTLMALGTFPESHELHMGMPGMHGTVSAVGALQRSDLLIAIGSRFDDRVTGDVDTFAPDAKIIHADIDPAEIGKIKQVEVPIVGDAREVLARLLETTKASKAETEDISEWVDYLKGLKARFPRGYDEQPGDLLAPQFVIETLSKEVGPDAIYCAGVGQHQMWAAQFVDFEKPRTWLNSGGLGTMGYAVPAALGAKAGAPDKEVWAIDGDGCFQMTNQELTTAAVEGFPIKIALINNGNLGMVRQWQTLFYEGRYSNTKLRNQGEYMPDFVTLSEGLGCVAIRVTKAEEVLPAIQKAREINDRPVVIDFIVGEDAQVWPMVSAGSSNSDIQYALGLRPFFDGDESAAEDPADIHEAVSDIDAAVESTEA

SEQ ID NO: 48 - protein, 626 aa, Artificial Sequence
  acetohydroxy acid synthase variant
MNVAASQQPTPATVASRGRSAAPERMTGAKAIVRSLEELNADIVFGIPGGAVLPVYDPLYSSTKVRHVLVRHEQGAGHAATGYAQVTGRVGVCIATSGPGATNLVTPIADANLDSVPMVAITGQVGSGLLGTDAFFEADIRGITMPVTKHNFMVTNPNDIPQALAEAFHLAITGRPGPVLVDIPKDVQNAELDFVWPPKIDLPGYRPVSTPHARQIEQAVKLIGEAKKPVLYVGGGVIKADAHEELRAFAEYTGIPVVTTLMALGTFPESHELHMGMPGMHGTVSAVGALQRSDLLIAIGSRFDDRVTGDVDTFAPDAKIIHADIDPAEIGKIKQVEVPIVGDAREVLARLLETTKASKAETEDISEWVDYLKGLKARFPRGYDEQPGDLLAPQFVIETLSKEVGPDAIYCAGVGQHQMWAAQFVDFEKPRTWLNSGGLGTMGYAVPAALGAKAGAPDKEVWAIDGDGCFQMTNQELTTAAVEGFPIKIALINNGNLGMVRQWQTLFYEGRYSNTKLRNQGEYMPDFVTLSEGLGCVAIRVTKAEEVLPAIQKAREINDRPVVIDFIVGEDAQVWPMVSAGSSNSDIQYALGLRPFFDGDESAAEDPADIHEAVSDIDAAVESTEA

SEQ ID NO: 49 - protein, 626 aa, Artificial Sequence
  acetohydroxy acid synthase variant
MNVAASQQPTPATVASRGRSAAPERMTGAKAIVRSLEELNADIVFGIPGGAVLPVYDPLYSSTKVRHVLVRHEQGAGHAATGYAQVTGRVGVCIATSGPGATNLVTPIADANLDSVPMVAITGQVGSGLLGTDAFSEADIRGITMPVTKHNFMVTNPNDIPQALAEAFHLAITGRPGPVLVDIPKDVQNAELDFVWPPKIDLPGYRPVSTPHARQIEQAVKLIGEAKKPVLYVGGGVIKADAHEELRAFAEYTGIPVVTTLMALGTFPESHELHMGMPGMHGTVSAVGALQRSDLLIAIGSRFDDRVTGDVDTFAPDAKIIHADIDPAEIGKIKQVEVPIVGDAREVLARLLETTKASKAETEDISEWVDYLKGLKARFPRGYDEQPGDLLAPQFVIETLSKEVGPDAIYCAGVGQHQMWAAQFVDFEKPRTWLNSGGLGTMGYAVPAALGAKAGAPDKEVWAIDGDGCFQMTNQELTTAAVEGFPIKIALINNGNLGMVRQWQTLFYEGRYSNTKLRNQGEYMPDFVTLSEGLGCVAIRVTKAEEVLPAIQKAREINDRPVVIDFIVGEDAQVWPMVSAGSSNSDIQYALGLRPFFDGDESAAEDPADIHEAVSDIDAAVESTEA

SEQ ID NO: 50 - protein, 626 aa, Artificial Sequence
  acetohydroxy acid synthase variant
MNVAASQQPTPATVASRGRSAAPERMTGAKAIVRSLEELNADIVFGIPGGAVLPVYDPLYSSTKVRHVLVRHEQGAGHAATGYAQVTGRVGVCIATSGPGATNLVTPIADANLDSVPMVAITGQVGSGLLGTDAFYEADIRGITMPVTKHNFMVTNPNDIPQALAEAFHLAITGRPGPVLVDIPKDVQNAELDFVWPPKIDLPGYRPVSTPHARQIEQAVKLIGEAKKPVLYVGGGVIKADAHEELRAFAEYTGIPVVTTLMALGTFPESHELHMGMPGMHGTVSAVGALQRSDLLIAIGSRFDDRVTGDVDTFAPDAKIIHADIDPAEIGKIKQVEVPIVGDAREVLARLLETTKASKAETEDISEWVDYLKGLKARFPRGYDEQPGDLLAPQFVIETLSKEVGPDAIYCAGVGQHQMWAAQFVDFEKPRTWLNSGGLGTMGYAVPAALGAKAGAPDKEVWAIDGDGCFQMTNQELTTAAVEGFPIKIALINNGNLGMVRQWQTLFYEGRYSNTKLRNQGEYMPDFVTLSEGLGCVAIRVTKAEEVLPAIQKAREINDRPVVIDFIVGEDAQVWPMVSAGSSNSDIQYALGLRPFFDGDESAAEDPADIHEAVSDIDAAVESTEA

SEQ ID NO: 51 - protein, 626 aa, Artificial Sequence
  acetohydroxy acid synthase variant
MNVAASQQPTPATVASRGRSAAPERMTGAKAIVRSLEELNADIVFGIPGGAVLPVYDPLYSSTKVRHVLVRHEQGAGHAATGYAQVTGRVGVCIATSGPGATNLVTPIADANLDSVPMVAITGQVGSGLLGTDAFCEADIRGITMPVTKHNFMVTNPNDIPQALAEAFHLAITGRPGPVLVDIPKDVQNAELDFVWPPKIDLPGYRPVSTPHARQIEQAVKLIGEAKKPVLYVGGGVIKADAHEELRAFAEYTGIPVVTTLMALGTFPESHELHMGMPGMHGTVSAVGALQRSDLLIAIGSRFDDRVTGDVDTFAPDAKIIHADIDPAEIGKIKQVEVPIVGDAREVLARLLETTKASKAETEDISEWVDYLKGLKARFPRGYDEQPGDLLAPQFVIETLSKEVGPDAIYCAGVGQHQMWAAQFVDFEKPRTWLNSGGLGTMGYAVPAALGAKAGAPDKEVWAIDGDGCFQMTNQELTTAAVEGFPIKIALINNGNLGMVRQWQTLFYEGRYSNTKLRNQGEYMPDFVTLSEGLGCVAIRVTKAEEVLPAIQKAREINDRPVVIDFIVGEDAQVWPMVSAGSSNSDIQYALGLRPFFDGDESAAEDPADIHEAVSDIDAAVESTEA

SEQ ID NO: 52 - protein, 626 aa, Artificial Sequence
  acetohydroxy acid synthase variant
MNVAASQQPTPATVASRGRSAAPERMTGAKAIVRSLEELNADIVFGIPGGAVLPVYDPLYSSTKVRHVLVRHEQGAGHAATGYAQVTGRVGVCIATSGPGATNLVTPIADANLDSVPMVAITGQVGSGLLGTDAFPEADIRGITMPVTKHNFMVTNPNDIPQALAEAFHLAITGRPGPVLVDIPKDVQNAELDFVWPPKIDLPGYRPVSTPHARQIEQAVKLIGEAKKPVLYVGGGVIKADAHEELRAFAEYTGIPVVTTLMALGTFPESHELHMGMPGMHGTVSAVGALQRSDLLIAIGSRFDDRVTGDVDTFAPDAKIIHADIDPAEIGKIKQVEVPIVGDAREVLARLLETTKASKAETEDISEWVDYLKGLKARFPRGYDEQPGDLLAPQFVIETLSKEVGPDAIYCAGVGQHQMWAAQFVDFEKPRTWLNSGGLGTMGYAVPAALGAKAGAPDKEVWAIDGDGCFQMTNQELTTAAVEGFPIKIALINNGNLGMVRQWQTLFYEGRYSNTKLRNQGEYMPDFVTLSEGLGCVAIRVTKAEEVLPAIQKAREINDRPVVIDFIVGEDAQVWPMVSAGSSNSDIQYALGLRPFFDGDESAAEDPADIHEAVSDIDAAVESTEA

SEQ ID NO: 53 - protein, 626 aa, Artificial Sequence
  acetohydroxy acid synthase variant
MNVAASQQPTPATVASRGRSAAPERMTGAKAIVRSLEELNADIVFGIPGGAVLPVYDPLYSSTKVRHVLVRHEQGAGHAATGYAQVTGRVGVCIATSGPGATNLVTPIADANLDSVPMVAITGQVGSGLLGTDAFHEADIRGITMPVTKHNFMVTNPNDIPQALAEAFHLAITGRPGPVLVDIPKDVQNAELDFVWPPKIDLPGYRPVSTPHARQIEQAVKLIGEAKKPVLYVGGGVIKADAHEELRAFAEYTGIPVVTTLMALGTFPESHELHMGMPGMHGTVSAVGALQRSDLLIAIGSRFDDRVTGDVDTFAPDAKIIHADIDPAEIGKIKQVEVPIVGDAREVLARLLETTKASKAETEDISEWVDYLKGLKARFPRGYDEQPGDLLAPQFVIETLSKEVGPDAIYCAGVGQHQMWAAQFVDFEKPRTWLNSGGLGTMGYAVPAALGAKAGAPDKEVWAIDGDGCFQMTNQELTTAAVEGFPIKIALINNGNLGMVRQWQTLFYEGRYSNTKLRNQGEYMPDFVTLSEGLGCVAIRVTKAEEVLPAIQKAREINDRPVVIDFIVGEDAQVWPMVSAGSSNSDIQYALGLRPFFDGDESAAEDPADIHEAVSDIDAAVESTEA

SEQ ID NO: 54 - protein, 626 aa, Artificial Sequence
  acetohydroxy acid synthase variant
MNVAASQQPTPATVASRGRSAAPERMTGAKAIVRSLEELNADIVFGIPGGAVLPVYDPLYSSTKVRHVLVRHEQGAGHAATGYAQVTGRVGVCIATSGPGATNLVTPIADANLDSVPMVAITGQVGSGLLGTDAFLEADIRGITMPVTKHNFMVTNPNDIPQALAEAFHLAITGRPGPVLVDIPKDVQNAELDFVWPPKIDLPGYRPVSTPHARQIEQAVKLIGEAKKPVLYVGGGVIKADAHEELRAFAEYTGIPVVTTLMALGTFPESHELHMGMPGMHGTVSAVGALQRSDLLIAIGSRFDDRVTGDVDTFAPDAKIIHADIDPAEIGKIKQVEVPIVGDAREVLARLLETTKASKAETEDISEWVDYLKGLKARFPRGYDEQPGDLLAPQFVIETLSKEVGPDAIYCAGVGQHQMWAAQFVDFEKPRTWLNSGGLGTMGYAVPAALGAKAGAPDKEVWAIDGDGCFQMTNQELTTAAVEGFPIKIALINNGNLGMVRQWQTLFYEGRYSNTKLRNQGEYMPDFVTLSEGLGCVAIRVTKAEEVLPAIQKAREINDRPVVIDFIVGEDAQVWPMVSAGSSNSDIQYALGLRPFFDGDESAAEDPADIHEAVSDIDAAVESTEA

SEQ ID NO: 55 - protein, 626 aa, Artificial Sequence
  acetohydroxy acid synthase variant
MNVAASQQPTPATVASRGRSAAPERMTGAKAIVRSLEELNADIVFGIPGGAVLPVYDPLYSSTKVRHVLVRHEQGAGHAATGYAQVTGRVGVCIATSGPGATNLVTPIADANLDSVPMVAITGQVGSGLLGTDAFIEADIRGITMPVTKHNFMVTNPNDIPQALAEAFHLAITGRPGPVLVDIPKDVQNAELDFVWPPKIDLPGYRPVSTPHARQIEQAVKLIGEAKKPVLYVGGGVIKADAHEELRAFAEYTGIPVVTTLMALGTFPESHELHMGMPGMHGTVSAVGALQRSDLLIAIGSRFDDRVTGDVDTFAPDAKIIHADIDPAEIGKIKQVEVPIVGDAREVLARLLETTKASKAETEDISEWVDYLKGLKARFPRGYDEQPGDLLAPQFVIETLSKEVGPDAIYCAGVGQHQMWAAQFVDFEKPRTWLNSGGLGTMGYAVPAALGAKAGAPDKEVWAIDGDGCFQMTNQELTTAAVEGFPIKIALINNGNLGMVRQWQTLFYEGRYSNTKLRNQGEYMPDFVTLSEGLGCVAIRVTKAEEVLPAIQKAREINDRPVVIDFIVGEDAQVWPMVSAGSSNSDIQYALGLRPFFDGDESAAEDPADIHEAVSDIDAAVESTEA

SEQ ID NO: 56 - protein, 626 aa, Artificial Sequence
  acetohydroxy acid synthase variant
MNVAASQQPTPATVASRGRSAAPERMTGAKAIVRSLEELNADIVFGIPGGAVLPVYDPLYSSTKVRHVLVRHEQGAGHAATGYAQVTGRVGVCIATSGPGATNLVTPIADANLDSVPMVAITGQVGSGLLGTDAFTEADIRGITMPVTKHNFMVTNPNDIPQALAEAFHLAITGRPGPVLVDIPKDVQNAELDFVWPPKIDLPGYRPVSTPHARQIEQAVKLIGEAKKPVLYVGGGVIKADAHEELRAFAEYTGIPVVTTLMALGTFPESHELHMGMPGMHGTVSAVGALQRSDLLIAIGSRFDDRVTGDVDTFAPDAKIIHADIDPAEIGKIKQVEVPIVGDAREVLARLLETTKASKAETEDISEWVDYLKGLKARFPRGYDEQPGDLLAPQFVIETLSKEVGPDAIYCAGVGQHQMWAAQFVDFEKPRTWLNSGGLGTMGYAVPAALGAKAGAPDKEVWAIDGDGCFQMTNQELTTAAVEGFPIKIALINNGNLGMVRQWQTLFYEGRYSNTKLRNQGEYMPDFVTLSEGLGCVAIRVTKAEEVLPAIQKAREINDRPVVIDFIVGEDAQVWPMVSAGSSNSDIQYALGLRPFFDGDESAAEDPADIHEAVSDIDAAVESTEA

SEQ ID NO: 57 - protein, 626 aa, Artificial Sequence
  acetohydroxy acid synthase variant
MNVAASQQPTPATVASRGRSAAPERMTGAKAIVRSLEELNADIVFGIPGGAVLPVYDPLYSSTKVRHVLVRHEQGAGHAATGYAQVTGRVGVCIATSGPGATNLVTPIADANLDSVPMVAITGQVGSGLLGTDAFKEADIRGITMPVTKHNFMVTNPNDIPQALAEAFHLAITGRPGPVLVDIPKDVQNAELDFVWPPKIDLPGYRPVSTPHARQIEQAVKLIGEAKKPVLYVGGGVIKADAHEELRAFAEYTGIPVVTTLMALGTFPESHELHMGMPGMHGTVSAVGALQRSDLLIAIGSRFDDRVTGDVDTFAPDAKIIHADIDPAEIGKIKQVEVPIVGDAREVLARLLETTKASKAETEDISEWVDYLKGLKARFPRGYDEQPGDLLAPQFVIETLSKEVGPDAIYCAGVGQHQMWAAQFVDFEKPRTWLNSGGLGTMGYAVPAALGAKAGAPDKEVWAIDGDGCFQMTNQELTTAAVEGFPIKIALINNGNLGMVRQWQTLFYEGRYSNTKLRNQGEYMPDFVTLSEGLGCVAIRVTKAEEVLPAIQKAREINDRPVVIDFIVGEDAQVWPMVSAGSSNSDIQYALGLRPFFDGDESAAEDPADIHEAVSDIDAAVESTEA

SEQ ID NO: 58 - protein, 626 aa, Artificial Sequence
  acetohydroxy acid synthase variant
MNVAASQQPTPATVASRGRSAAPERMTGAKAIVRSLEELNADIVFGIPGGAVLPVYDPLYSSTKVRHVLVRHEQGAGHAATGYAQVTGRVGVCIATSGPGATNLVTPIADANLDSVPMVAITGQVGSGLLGTDAFVEADIRGITMPVTKHNFMVTNPNDIPQALAEAFHLAITGRPGPVLVDIPKDVQNAELDFVWPPKIDLPGYRPVSTPHARQIEQAVKLIGEAKKPVLYVGGGVIKADAHEELRAFAEYTGIPVVTTLMALGTFPESHELHMGMPGMHGTVSAVGALQRSDLLIAIGSRFDDRVTGDVDTFAPDAKIIHADIDPAEIGKIKQVEVPIVGDAREVLARLLETTKASKAETEDISEWVDYLKGLKARFPRGYDEQPGDLLAPQFVIETLSKEVGPDAIYCAGVGQHQMWAAQFVDFEKPRTWLNSGGLGTMGYAVPAALGAKAGAPDKEVWAIDGDGCFQMTNQELTTAAVEGFPIKIALINNGNLGMVRQWQTLFYEGRYSNTKLRNQGEYMPDFVTLSEGLGCVAIRVTKAEEVLPAIQKAREINDRPVVIDFIVGEDAQVWPMVSAGSSNSDIQYALGLRPFFDGDESAAEDPADIHEAVSDIDAAVESTEA

SEQ ID NO: 59 - protein, 626 aa, Artificial Sequence
  acetohydroxy acid synthase variant
MNVAASQQPTPATVASRGRSAAPERMTGAKAIVRSLEELNADIVFGIPGGAVLPVYDPLYSSTKVRHVLVRHEQGAGHAATGYAQVTGRVGVCIATSGPGATNLVTPIADANLDSVPMVAITGQVGSGLLGTDAFAEADIRGITMPVTKHNFMVTNPNDIPQALAEAFHLAITGRPGPVLVDIPKDVQNAELDFVWPPKIDLPGYRPVSTPHARQIEQAVKLIGEAKKPVLYVGGGVIKADAHEELRAFAEYTGIPVVTTLMALGTFPESHELHMGMPGMHGTVSAVGALQRSDLLIAIGSRFDDRVTGDVDTFAPDAKIIHADIDPAEIGKIKQVEVPIVGDAREVLARLLETTKASKAETEDISEWVDYLKGLKARFPRGYDEQPGDLLAPQFVIETLSKEVGPDAIYCAGVGQHQMWAAQFVDFEKPRTWLNSGGLGTMGYAVPAALGAKAGAPDKEVWAIDGDGCFQMTNQELTTAAVEGFPIKIALINNGNLGMVRQWQTLFYEGRYSNTKLRNQGEYMPDFVTLSEGLGCVAIRVTKAEEVLPAIQKAREINDRPVVIDFIVGEDAQVWPMVSAGSSNSDIQYALGLRPFFDGDESAAEDPADIHEAVSDIDAAVESTEA

SEQ ID NO: 60 - protein, 626 aa, Artificial Sequence
  acetohydroxy acid synthase variant
MNVAASQQPTPATVASRGRSAAPERMTGAKAIVRSLEELNADIVFGIPGGAVLPVYDPLYSSTKVRHVLVRHEQGAGHAATGYAQVTGRVGVCIATSGPGATNLVTPIADANLDSVPMVAITGQVGSGLLGTDAFDEADIRGITMPVTKHNFMVTNPNDIPQALAEAFHLAITGRPGPVLVDIPKDVQNAELDFVWPPKIDLPGYRPVSTPHARQIEQAVKLIGEAKKPVLYVGGGVIKADAHEELRAFAEYTGIPVVTTLMALGTFPESHELHMGMPGMHGTVSAVGALQRSDLLIAIGSRFDDRVTGDVDTFAPDAKIIHADIDPAEIGKIKQVEVPIVGDAREVLARLLETTKASKAETEDISEWVDYLKGLKARFPRGYDEQPGDLLAPQFVIETLSKEVGPDAIYCAGVGQHQMWAAQFVDFEKPRTWLNSGGLGTMGYAVPAALGAKAGAPDKEVWAIDGDGCFQMTNQELTTAAVEGFPIKIALINNGNLGMVRQWQTLFYEGRYSNTKLRNQGEYMPDFVTLSEGLGCVAIRVTKAEEVLPAIQKAREINDRPVVIDFIVGEDAQVWPMVSAGSSNSDIQYALGLRPFFDGDESAAEDPADIHEAVSDIDAAVESTEA

SEQ ID NO: 61 - protein, 626 aa, Artificial Sequence
  acetohydroxy acid synthase variant
MNVAASQQPTPATVASRGRSAAPERMTGAKAIVRSLEELNADIVFGIPGGAVLPVYDPLYSSTKVRHVLVRHEQGAGHAATGYAQVTGRVGVCIATSGPGATNLVTPIADANLDSVPMVAITGQVGSGLLGTDAFEEADIRGITMPVTKHNFMVTNPNDIPQALAEAFHLAITGRPGPVLVDIPKDVQNAELDFVWPPKIDLPGYRPVSTPHARQIEQAVKLIGEAKKPVLYVGGGVIKADAHEELRAFAEYTGIPVVTTLMALGTFPESHELHMGMPGMHGTVSAVGALQRSDLLIAIGSRFDDRVTGDVDTFAPDAKIIHADIDPAEIGKIKQVEVPIVGDAREVLARLLETTKASKAETEDISEWVDYLKGLKARFPRGYDEQPGDLLAPQFVIETLSKEVGPDAIYCAGVGQHQMWAAQFVDFEKPRTWLNSGGLGTMGYAVPAALGAKAGAPDKEVWAIDGDGCFQMTNQELTTAAVEGFPIKIALINNGNLGMVRQWQTLFYEGRYSNTKLRNQGEYMPDFVTLSEGLGCVAIRVTKAEEVLPAIQKAREINDRPVVIDFIVGEDAQVWPMVSAGSSNSDIQYALGLRPFFDGDESAAEDPADIHEAVSDIDAAVESTEA

SEQ ID NO: 62 - protein, 626 aa, Artificial Sequence
  acetohydroxy acid synthase variant
MNVAASQQPTPATVASRGRSAAPERMTGAKAIVRSLEELNADIVFGIPGGAVLPVYDPLYSSTKVRHVLVRHEQGAGHAATGYAQVTGRVGVCIATSGPGATNLVTPIADANLDSVPMVAITGQVGSGLLGTDAFGEADIRGITMPVTKHNFMVTNPNDIPQALAEAFHLAITGRPGPVLVDIPKDVQNAELDFVWPPKIDLPGYRPVSTPHARQIEQAVKLIGEAKKPVLYVGGGVIKADAHEELRAFAEYTGIPVVTTLMALGTFPESHELHMGMPGMHGTVSAVGALQRSDLLIAIGSRFDDRVTGDVDTFAPDAKIIHADIDPAEIGKIKQVEVPIVGDAREVLARLLETTKASKAETEDISEWVDYLKGLKARFPRGYDEQPGDLLAPQFVIETLSKEVGPDAIYCAGVGQHQMWAAQFVDFEKPRTWLNSGGLGTMGYAVPAALGAKAGAPDKEVWAIDGDGCFQMTNQELTTAAVEGFPIKIALINNGNLGMVRQWQTLFYEGRYSNTKLRNQGEYMPDFVTLSEGLGCVAIRVTKAEEVLPAIQKAREINDRPVVIDFIVGEDAQVWPMVSAGSSNSDIQYALGLRPFFDGDESAAEDPADIHEAVSDIDAAVESTEA

SEQ ID NO: 63 - protein, 626 aa, Artificial Sequence
  acetohydroxy acid synthase variant
MNVAASQQPTPATVASRGRSAAPERMTGAKAIVRSLEELNADIVFGIPGGAVLPVYDPLYSSTKVRHVLVRHEQGAGHAATGYAQVTGRVGVCIATSGPGATNLVTPIADANLDSVPMVAITGQVGSGLLGTDAFWEADIRGITMPVTKHNFMVTNPNDIPQALAEAFHLAITGRPGPVLVDIPKDVQNAELDFVWPPKIDLPGYRPVSTPHARQIEQAVKLIGEAKKPVLYVGGGVIKADAHEELRAFAEYTGIPVVTTLMALGTFPESHELHMGMPGMHGTVSAVGALQRSDLLIAIGSRFDDRVTGDVDTFAPDAKIIHADIDPAEIGKIKQVEVPIVGDAREVLARLLETTKASKAETEDISEWVDYLKGLKARFPRGYDEQPGDLLAPQFVIETLSKEVGPDAIYCAGVGQHQMWAAQFVDFEKPRTWLNSGGLGTMGYAVPAALGAKAGAPDKEVWAIDGDGCFQMTNQELTTAAVEGFPIKIALINNGNLGMVRQWQTLFYEGRYSNTKLRNQGEYMPDFVTLSEGLGCVAIRVTKAEEVLPAIQKAREINDRPVVIDFIVGEDAQVWPMVSAGSSNSDIQYALGLRPFFDGDESAAEDPADIHEAVSDIDAAVESTEA

SEQ ID NO: 64 - DNA, 38 bp, Artificial Sequence
  primer
tcgagctcggtacccgctcactgaggacgcttttgcac

SEQ ID NO: 65 - DNA, 24 bp, Artificial Sequence
  primer
gaagagcgcgatgatgatgcacac

SEQ ID NO: 66 - DNA, 23 bp, Artificial Sequence
  primer
tgatgatgcacacctgatcgtgg

SEQ ID NO: 67 - DNA, 38 bp, Artificial Sequence
  primer
ggggatcctctagaggacaaggttttggaagatgctcg

SEQ ID NO: 68 - DNA, 20 bp, Artificial Sequence
  primer
agcgcgatgatgatgcacac

SEQ ID NO: 69 - DNA, 20 bp, Artificial Sequence
  primer
catctggcttggaagtggaa

SEQ ID NO: 70 - DNA, 20 bp, Artificial Sequence
  primer
atgacctcagcatctgcccc

SEQ ID NO: 71 - DNA, 20 bp, Artificial Sequence
  primer
tccgcctcgaaagggactaa

SEQ ID NO: 72 - DNA, 35 bp, Artificial Sequence
  primer
tcgagctcggtacccatgagtgaaacatacgtgtc

SEQ ID NO: 73 - DNA, 20 bp, Artificial Sequence
  primer
ggtactctgacagcgtgatg

SEQ ID NO: 74 - DNA, 22 bp, Artificial Sequence
  primer
cacgctggcagagtacctcaag

SEQ ID NO: 75 - DNA, 35 bp, Artificial Sequence
  primer
ggggatcctctagagtggatgcacagtgggttgac

SEQ ID NO: 76 - DNA, 24 bp, Artificial Sequence
  primer
gtaacgaacttggggtcattgagt

SEQ ID NO: 77 - DNA, 22 bp, Artificial Sequence
  primer
atgagtgaaacatacgtgtctg

SEQ ID NO: 78 - DNA, 23 bp, Artificial Sequence
  primer
ttaggtcaagtattcgtactcag